European Patent Application EP 4 567 041 A1, published June 11, 2025. Title: A Method for the Purification of Proteins Fused to Multiprotein Complexes by Metal Affinity Precipitation, and Uses Thereof. Applicant: Lock and Key Biosciences GmbH. Application EP. The sequence listing filed with the application follows.

SEQUENCE LISTING (4 sequences)

SEQ ID NO: 1 - protein, 6 aa, synthetic construct
HHHHHH

SEQ ID NO: 2 - protein, 6 aa, synthetic construct
HQHQHQ

SEQ ID NO: 3 - protein, 12 aa, synthetic construct
HNHNHNHNHNHN

SEQ ID NO: 4 - protein, 19 aa, synthetic construct
KDHLIHNVHKEEHAHAHNK